European Patent Application EP 4 737 583 A1, published May 6, 2026. Title: 目的タンパク質の生産方法. Applicant: 花王株式会社. The sequence listing filed with the application follows.

SEQUENCE LISTING (101 sequences)

SEQ ID NO: 1 - protein, 245 aa, Escherichia coli
AEAAKPATAADSKAAFKNDDQKSAYALGASLGRYMENSLKEQEKLGIKLDKDQLIAGVQDAFADKSKLSDQEIEQTLQAFEARVKSSAQAKMEKDAADNEAKGKEYREKFAKEKGVKTSSTGLVYQVVEAGKGEAPKDSDTVVVNYKGTLIDGKEFDNSYTRGEPLSFRLDGVIPGWTEGLKNIKKGGKIKLVIPPELAYGKAGVPGIPPNSTLVFDVELLDVKPAPKADAKPEADAKAADSAKK

SEQ ID NO: 2 - protein, 233 aa, Lelliottia amnigena
AFKNDDQKSAYALGASLGRYMENSLKEQEKLGIKLDKDQLIAGVQDAFADKSKLSDQEIEQTLQAFEARVKGAAQGKMEKDAKDNEAKGKAYRDTFAKEKGVKTSSTGLLYKVEKAGTGDAPKDSDTVVVNYKGTLIDGKEFDNSYTRGEPLSFRLDGVIPGWTEGLKNIKKGGKIQLVIPPDLAYGKTGVPGIPANSTLVFDVELLDIKPAPKADAKSAAAEDDKAADAAKK

SEQ ID NO: 3 - protein, 236 aa, Klebsiella quasipneumoniae
AFKNDDQKSAYALGASLGRYMENSLKEQEKLGIKLDKAQLIAGVQDAFADKSKLSDQEIEQTLQAFETRVKTAAQQKMQNHATENETKGKAFRDSFAKEKGVKTSKTGLLYKVEKEGTGDAPKDSDTVVVNYKGTLIDGKEFDNSYTRGEPLSFRLDGVIPGWTEGLKNIKKGGKIKLVIPPDLAYGKTGVPGIPANSTLVFDVELLDIKPAPKADAQPEAAGDAKAADAKADAKK

SEQ ID NO: 4 - protein, 233 aa, Erwinia sp. B116
AFKNDDQQSAYALGASLGRYMENSLKEQEKLGIALDKNQLIAGVQDAFAGKSKLTDQEIEQTLQSFEGRVKGAAQAKMEKDAKENTAKGEAYAAKFAKEKDVKKTESGLLYLVEKAGAGESPKDSDTVVVNYKGTLVDGTEFDNSYTRGEPLSFRLDGVIPGWTEGLKQVKKGGKIKLVIPPALAYGQNGVPGIPANSTLVFEVELLDIKPAAKADEKAEQPAAAAADKAKAQ

SEQ ID NO: 5 - protein, 230 aa, Pantoea sp. Nvir
FFKNEDQQSAYALGASLARYMNNSLEEQKKLGIKLDKQQLLEGVQDMFAGKSKLSEQRIEQILHGLESRVKGATQEKMEKEAKENADKGIAFANKFAKESGVKKTESGLLYKIEKEGSGDPPQDDTTVVVHYKGMLINGTEFDNSYTRGQPLSLHLQGIIPGWTEGLKHVKKGGKIKLVIPPQLAYGKNNVPGIPINSTLVFDIELLDIKTSPKKDDKARALVTEMNKFK

SEQ ID NO: 6 - protein, 156 aa, Methanococcus jannaschii
INLIKKGDYVKVDYILEVDGKVIDTSIEEVAKENKIYYPEREYEPIGFIVGNGELIEGFEEAVIGMEVGEEKTVTIPPEKGYGLRDERLIQEIPKEMFADADFEPQEGMLILASGIPAKIIKVTDDTVTLDFNHELAGKELKFTIKVRDVQPAESE

SEQ ID NO: 7 - DNA, 31 bp, synthetic construct
  source 1..31: mol_type = other DNA
gatccccgggaattcctgttataaaaaaagg

SEQ ID NO: 8 - DNA, 27 bp, synthetic construct
  source 1..27: mol_type = other DNA
atgatgttaagaaagaaaacaaagcag

SEQ ID NO: 9 - DNA, 38 bp, synthetic construct
  source 1..38: mol_type = other DNA
gaattcccggggatctaagaaaagtgattctgggagag

SEQ ID NO: 10 - DNA, 36 bp, synthetic construct
  source 1..36: mol_type = other DNA
ctttcttaacatcatagtagttcacctccttttccc

SEQ ID NO: 11 - DNA, 20 bp, synthetic construct
  source 1..20: mol_type = other DNA
agtagttcacctccttttcc

SEQ ID NO: 12 - DNA, 54 bp, synthetic construct
  source 1..54: mol_type = other DNA
aggaggtgaactacttaatctattaaactagttatagggttatctaaaggtctg

SEQ ID NO: 13 - DNA, 39 bp, synthetic construct
  source 1..39: mol_type = other DNA
taatctattaaactagttatagggttatctaaaggtctg

SEQ ID NO: 14 - DNA, 37 bp, synthetic construct
  source 1..37: mol_type = other DNA
tagtttaatagattaagccgaagcttcccctacatgg

SEQ ID NO: 15 - DNA, 38 bp, synthetic construct
  source 1..38: mol_type = other DNA
aggaggtgaactactatgaaaaagatgttgatgttagc

SEQ ID NO: 16 - DNA, 38 bp, synthetic construct
  source 1..38: mol_type = other DNA
tagtttaatagattatttagaattgcttgaagatgaag

SEQ ID NO: 17 - DNA, 38 bp, synthetic construct
  source 1..38: mol_type = other DNA
aggaggtgaactactatgaagaaaatcgcaatagcagc

SEQ ID NO: 18 - protein, 292 aa, Bacillus subtilis
MKKIAIAAITATSILALSACSSGDKEVIAKTDAGDVTKGELYTNMKKTAGASVLTQLVQEKVLDKKYKVSDKEIDNKLKEYKTQLGDQYTALEKQYGKDYLKEQVKYELLTQKAAKDNIKVTDADIKEYWEGLKGKIRASHILVADKKTAEEVEKKLKKGEKFEDLAKEYSTDSSASKGGDLGWFAKEGQMDETFSKAAFKLKTGEVSDPVKTQYGYHIIKKTEERGKYDDMKKELKSEVLEQKLNDNAAVQEAVQKVMKKADIEVKDKDLKDTFNTSSTSNSTSSSSSNSK

SEQ ID NO: 19 - protein, 876 aa, Bacillus subtilis
ATGAAGAAAATCGCAATAGCAGCTATCACTGCTACAAGCATCCTCGCTCTCAGTGCTTGCAGCAGCGGCGACAAAGAAGTTATCGCAAAAACAGACGCAGGCGATGTCACAAAAGGCGAGCTTTACACAAACATGAAGAAAACAGCTGGCGCAAGCGTACTGACACAGCTAGTGCAAGAAAAAGTATTGGACAAGAAGTATAAAGTTTCGGATAAAGAAATTGACAACAAGCTGAAAGAATACAAAACGCAGCTTGGCGATCAATATACTGCCCTCGAAAAGCAATATGGCAAAGATTACCTGAAAGAACAAGTAAAATATGAATTGCTGACACAAAAAGCGGCTAAAGATAACATCAAAGTAACAGACGCCGATATCAAAGAGTACTGGGAAGGCTTAAAAGGCAAAATCCGTGCAAGCCACATCCTTGTTGCTGATAAAAAGACAGCTGAAGAAGTAGAGAAAAAGCTGAAAAAAGGCGAGAAGTTTGAAGACCTTGCGAAAGAATACTCAACAGACAGCTCTGCTTCAAAAGGCGGGGATCTTGGCTGGTTCGCAAAAGAAGGCCAAATGGACGAAACATTCAGCAAAGCTGCATTCAAATTAAAAACAGGTGAAGTCAGTGATCCTGTCAAAACGCAATACGGCTACCATATCATTAAAAAGACAGAAGAACGCGGCAAATATGATGATATGAAAAAAGAACTGAAATCTGAAGTGCTTGAACAAAAATTAAATGACAACGCAGCTGTTCAGGAAGCTGTTCAAAAAGTCATGAAGAAGGCTGACATCGAAGTAAAAGATAAAGATCTGAAAGACACATTTAATACATCTTCAACAAGCAACAGCACTTCTTCATCTTCAAGCAATTCTAAA

SEQ ID NO: 20 - DNA, 22 bp, synthetic construct
  source 1..22: mol_type = other DNA
ccatgtaggggaagcttcggct

SEQ ID NO: 21 - DNA, 37 bp, synthetic construct
  source 1..37: mol_type = other DNA
ggggaagcttcggctgccccccaggtagtcgataaag

SEQ ID NO: 22 - DNA, 41 bp, synthetic construct
  source 1..41: mol_type = other DNA
aactagtttaatagattagttgctcaggattttaacgtagg

SEQ ID NO: 23 - DNA, 39 bp, synthetic construct
  source 1..39: mol_type = other DNA
ggggaagcttcggctgcgaaaggggacccgcacgtattg

SEQ ID NO: 24 - DNA, 40 bp, synthetic construct
  source 1..40: mol_type = other DNA
aactagtttaatagattacggcaggactttagcggaaagg

SEQ ID NO: 25 - DNA, 35 bp, synthetic construct
  source 1..35: mol_type = other DNA
ggggaagcttcggctcaagtttcagttgaaaccac

SEQ ID NO: 26 - DNA, 37 bp, synthetic construct
  source 1..37: mol_type = other DNA
aactagtttaatagattacgcctgctggttcatcagc

SEQ ID NO: 27 - DNA, 35 bp, synthetic construct
  source 1..35: mol_type = other DNA
ggggaagcttcggctgctgaagctgcaaaacctgc

SEQ ID NO: 28 - DNA, 44 bp, synthetic construct
  source 1..44: mol_type = other DNA
aactagtttaatagattattttttagcagaatctgcggctttcg

SEQ ID NO: 29 - protein, 408 aa, Escherichia coli
APQVVDKVAAVVNNGVVLESDVDGLMQSVKLNAAQARQQLPDDATLRHQIMERLIMDQIILQMGQKMGVKISDEQLDQAIANIAKQNNMTLDQMRSRLAYDGLNYNTYRNQIRKEMIISEVRNNEVRRRITILPQEVESLAQQVGNQNDASTELNLSHILIPLPENPTSDQVNEAESQARAIVDQARNGADFGKLAIAHSADQQALNGGQMGWGRIQELPGIFAQALSTAKKGDIVGPIRSGVGFHILKVNDLRGESKNISVTEVHARHILLKPSPIMTDEQARVKLEQIAADIKSGKTTFAAAAKEFSQDPGSANQGGDLGWATPDIFDPAFRDALTRLNKGQMSAPVHSSFGWHLIELLDTRNVDKTDAAQKDRAYRMLMNRKFSEEAASWMQEQRASAYVKILSN

SEQ ID NO: 30 - protein, 166 aa, Escherichia coli
AKGDPHVLLTTSAGNIELELDKQKAPVSVQNFVDYVNSGFYNNTTFHRVIPGFMIQGGGFTEQMQQKKPNPPIKNEADNGLRNTRGTIAMARTADKDSATSQFFINVADNAFLDHGQRDFGYAVFGKVVKGMDVADKISQVPTHDVGPYQNVPSKPVVILSAKVLP

SEQ ID NO: 31 - protein, 431 aa, Escherichia coli
QVSVETTQGLGRRVTITIAADSIETAVKSELVNVAKKVRIDGFRKGKVPMNIVAQRYGASVRQDVLGDLMSRNFIDAIIKEKINPAGAPTYVPGEYKLGEDFTYSVEFEVYPEVELQGLEAIEVEKPIVEVTDADVDGMLDTLRKQQATWKEKDGAVEAEDRVTIDFTGSVDGEEFEGGKASDFVLAMGQGRMIPGFEDGIKGHKAGEEFTIDVTFPEEYHAENLKGKAAKFAINLKKVEERELPELTAEFIKRFGVEDGSVEGLRAEVRKNMERELKSAIRNRVKSQAIEGLVKANDIDVPAALIDSEIDVLRRQAAQRFGGNEKQALELPRELFEEQAKRRVVVGLLLGEVIRTNELKADEERVKGLIEEMASAYEDPKEVIEFYSKNKELMDNMRNVALEEQAVEAVLAKAKVTEKETTFNELMNQQA

SEQ ID NO: 32 - DNA, 1224 bp, Escherichia coli
  source 1..1224: mol_type = genomic DNA
gccccccaggtagtcgataaagtcgcagccgtcgtcaataacggcgtcgtgctggaaagcgacgttgatggattaatgcagtcggtaaaactgaacgctgctcaggcaaggcagcaacttcctgatgacgcgacgctgcgccaccaaatcatggaacgtttgatcatggatcaaatcatcctgcagatggggcagaaaatgggagtgaaaatctccgatgagcagctggatcaggcgattgctaacatcgcgaaacagaacaacatgacgctggatcagatgcgcagccgtctggcttacgatggactgaactacaacacctatcgtaaccagatccgcaaagagatgattatctctgaagtgcgtaacaacgaggtgcgtcgtcgcatcaccatcctgccgcaggaagtcgaatccctggcgcagcaggtgggtaaccaaaacgacgccagcactgagctgaacctgagccacatcctgatcccgctgccggaaaacccgacctctgatcaggtgaacgaagcggaaagccaggcgcgcgccattgtcgatcaggcgcgtaacggcgctgatttcggtaagctggcgattgctcattctgccgaccagcaggcgctgaacggcggccagatgggctggggccgtattcaggagttgcccgggatcttcgcccaggcattaagcaccgcgaagaaaggcgacattgttggcccgattcgttccggcgttggcttccatattctgaaagttaacgacctgcgcggcgaaagcaaaaatatctcggtgaccgaagttcatgctcgccatattctgctgaaaccgtcgccgatcatgactgacgaacaggcccgtgtgaaactggaacagattgctgctgatatcaagagtggtaaaacgacttttgctgccgcagcgaaagagttctctcaggatccaggctctgctaaccagggcggcgatctcggctgggctacaccagatattttcgatccggccttccgtgacgccctgactcgcctgaacaaaggtcaaatgagtgcaccggttcactcttcattcggctggcatttaatcgaactgctggatacccgtaatgtcgataaaaccgacgctgcgcagaaagatcgtgcataccgcatgctgatgaaccgtaagttctcggaagaagcagcaagctggatgcaggaacaacgtgccagcgcctacgttaaaatcctgagcaac

SEQ ID NO: 33 - DNA, 498 bp, Escherichia coli
  source 1..498: mol_type = genomic DNA
gcgaaaggggacccgcacgtattgttgacaacctcagctggtaacatcgaactggagctggataaacaaaaagcgccagtgtctgtgcaaaactttgtcgattatgtgaacagcggtttttataacaacactacctttcaccgcgtcattcctggctttatgattcagggcggcggtttcaccgagcagatgcagcagaaaaaaccaaacccgccaatcaaaaatgaagccgataacggcctgcgcaacacgcgtggcaccatcgcgatggcacgtaccgctgacaaagacagcgccaccagccagttctttatcaacgttgccgataacgccttccttgaccatggtcagcgtgatttcggttacgcggtatttggtaaagtggtgaaaggcatggacgttgccgataagatttcccaggtgccgactcatgacgttggtccgtaccagaatgtgccgtcaaaaccggtagttatcctttccgctaaagtcctgccg

SEQ ID NO: 34 - DNA, 1293 bp, Escherichia coli
  source 1..1293: mol_type = genomic DNA
caagtttcagttgaaaccactcaaggccttggccgccgtgtaacgattactatcgctgctgacagcatcgagaccgctgttaaaagcgagctggtcaacgttgcgaaaaaagtacgtattgacggcttccgcaaaggcaaagtgccaatgaatatcgttgctcagcgttatggcgcgtctgtacgccaggacgttctgggtgacctgatgagccgtaacttcattgacgccatcattaaagaaaaaatcaatccggctggcgcaccgacttatgttccgggcgaatacaagctgggtgaagacttcacttactctgtagagtttgaagtttatccggaagttgaactgcagggtctggaagcgatcgaagttgaaaaaccgatcgttgaagtgaccgacgctgacgttgacggcatgctggatactctgcgtaaacagcaggcgacctggaaagaaaaagacggcgctgttgaagcagaagaccgcgtaaccatcgacttcaccggttctgtagacggcgaagagttcgaaggcggtaaagcgtctgatttcgtactggcgatgggccagggtcgtatgatcccgggctttgaagacggtatcaaaggccacaaagctggcgaagagttcaccatcgacgtgaccttcccggaagaataccacgcagaaaacctgaaaggtaaagcagcgaaattcgctatcaacctgaagaaagttgaagagcgtgaactgccggaactgactgcagaattcatcaaacgtttcggcgttgaagatggttccgtagaaggtctgcgcgctgaagtgcgtaaaaacatggagcgcgagctgaagagcgccatccgtaaccgcgttaagtctcaggcgatcgaaggtctggtaaaagctaacgacatcgacgtaccggctgcgctgatcgacagcgaaatcgacgttctgcgtcgccaggctgcacagcgtttcggtggcaacgaaaaacaagctctggaactgccgcgcgaactgttcgaagaacaggctaaacgccgcgtagttgttggcctgctgctgggcgaagttatccgcaccaacgagctgaaagctgacgaagagcgcgtgaaaggcctgatcgaagagatggcttctgcgtacgaagatccgaaagaagttatcgagttctacagcaaaaacaaagaactgatggacaacatgcgcaatgttgctctggaagaacaggctgttgaagctgtactggcgaaagcgaaagtgactgaaaaagaaaccactttcaacgagctgatgaaccagcaggcg

SEQ ID NO: 35 - DNA, 735 bp, Escherichia coli
  source 1..735: mol_type = genomic DNA
gctgaagctgcaaaacctgctacagctgctgacagcaaagcagcgttcaaaaatgacgatcagaaatcagcttatgcactgggtgcctcgctgggtcgttacatggaaaactctctaaaagaacaagaaaaactgggcatcaaactggataaagatcagctgatcgctggtgttcaggatgcatttgctgataagagcaaactctccgaccaagagatcgaacagactctacaagcattcgaagctcgcgtgaagtcttctgctcaggcgaagatggaaaaagacgcggctgataacgaagcaaaaggtaaagagtaccgcgagaaatttgccaaagagaaaggtgtgaaaacctcttcaactggtctggtttatcaggtagtagaagccggtaaaggcgaagcaccgaaagacagcgatactgttgtagtgaactacaaaggtacgctgatcgacggtaaagagttcgacaactcttacacccgtggtgaaccgctttctttccgtctggacggtgttatcccgggttggacagaaggtctgaagaacatcaagaaaggcggtaagatcaaactggttattccaccagaactggcttacggcaaagcgggtgttccggggatcccaccgaattctaccctggtgtttgacgtagagctgctggatgtgaaaccagcgccgaaggctgatgcaaagccggaagctgatgcgaaagccgcagattctgctaaaaaa

SEQ ID NO: 36 - protein, 119 aa, Saccharomyces cerevisiae
AGSLSDLEIGIIKRIPVEDCLIKAMPGDKVKVHYTGSLLESGTVFDSSYSRGSPIAFELGVGRVIKGWDQGVAGMCVGEKRKLQIPSSLAYGERGVPGVIPPSADLVFDVELVDVKSAA

SEQ ID NO: 37 - protein, 143 aa, Arabidopsis thaliana
ASPSESAKKNEKISEEATVESKAFSISVEKQTPDLDGLIVEELCMGNPNGKKAEPGKRVSVHYTGKLQGNGKIFDSTVGKSRYKFRLDAGKVIKGLDVGLNGMLVGGKRKLTIPPEMGYGAEGAGSIPPDSWLVFDVELLNVK

SEQ ID NO: 38 - protein, 459 aa, Homo sapiens
ATAEEMKATESGAQSAPLPMEGVDISPKQDEGVLKVIKREGTGTEMPMIGDRVFVHYTGWLLDGTKFDSSLDRKDKFSFDLGKGEVIKAWDIAIATMKVGEVCHITCKPEYAYGSAGSPPKIPPNATLVFEVELFEFKGEDLTEEEDGGIIRRIQTRGEGYAKPNEGAIVEVALEGYYKDKLFDQRELRFEIGEGENLDLPYGLERAIQRMEKGEHSIVYLKPSYAFGSVGKEKFQIPPNAELKYELHLKSFEKAKESWEMNSEEKLEQSTIVKERGTVYFKEGKYKQALLQYKKIVSWLEYESSFSNEEAQKAQALRLASHLNLAMCHLKLQAFSAAIESCNKALELDSNNEKGLFRRGEAHLAVNDFELARADFQKVLQLYPNNKAAKTQLAVCQQRIRRQLAREKKLYANMFERLAEEENKAKAEASSGDHPTDTEMKEEQKSNTAGSQSQVETEA

SEQ ID NO: 39 - protein, 370 aa, Homo sapiens
ASHPSPQAKPSNPSNPRVFFDVDIGGERVGRIVLELFADIVPKTAENFRALCTGEKGIGHTTGKPLHFKGCPFHRIIKKFMIQGGDFSNQNGTGGESIYGEKFEDENFHYKHDREGLLSMANAGRNTNGSQFFITTVPTPHLDGKHVVFGQVIKGIGVARILENVEVKGEKPAKLCVIAECGELKEGDDGGIFPKDGSGDSHPDFPEDADIDLKDVDKILLITEDLKNIGNTFFKSQNWEMAIKKYAEVLRYVDSSKAVIETADRAKLQPIALSCVLNIGACKLKMSNWQGAIDSCLEALELDPSNTKALYRRAQGWQGLKEYDQALADLKKAQGIAPEDKAIQAELLKVKQKIKAQKDKEKAVYAKMFA

SEQ ID NO: 40 - DNA, 699 bp, synthetic construct
  source 1..699: mol_type = other DNA
gcatttaaaaatgatgatcaaaaatctgcttatgcattgggggcttccctcggtcgttatatggaaaacagcctgaaagagcaagaaaagcttggaatcaagctggacaaagatcagctgattgccggcgttcaggacgcgttcgctgataaatcaaaattgagtgaccaggaaattgaacagacgcttcaagcttttgaagcgcgggtgaaaggtgccgcgcaaggaaaaatggagaaggatgcaaaggacaatgaagcgaagggaaaagcttaccgcgatacatttgccaaagaaaaaggcgtcaaaacaagctcaactggcctattatataaagtagaaaaggcgggaacaggtgatgcaccaaaagactctgatacggttgttgtgaattataagggcaccttgattgatgggaaggaatttgataattcctatacaagaggagagccgctgtcattcaggttagacggagtcatacccggctggactgaaggcttaaaaaacatcaaaaaaggagggaaaatccaacttgtcatcccgcctgatttagcatacggcaaaaccggtgtacctggcattccagcgaactcgacgctcgtgtttgatgttgagctgcttgatattaaaccggcgccgaaagcagacgcgaaaagcgccgctgctgaggacgataaggcagccgatgccgcaaaaaag

SEQ ID NO: 41 - DNA, 708 bp, synthetic construct
  source 1..708: mol_type = other DNA
gcctttaaaaatgatgatcagaaatcagcttatgctctaggggcatcgcttggccgctatatggaaaactccttaaaagaacaggaaaagctcggcatcaagcttgacaaagcgcagctgattgcaggtgtgcaagatgcatttgccgataaaagcaaattatctgatcaagaaattgaacaaacgctgcaagcgtttgaaacgagggtgaaaacggctgctcagcaaaaaatgcaaaatcatgcaacagaaaatgaaacaaaagggaaggcgttccgggattctttcgcaaaagagaaaggtgtaaagacttcaaagaccggtcttttatacaaagttgaaaaagaaggcactggcgacgcgcctaaagacagtgatacagttgttgtcaattataaaggaaccctcatagacggcaaggaatttgataacagctatacaagaggagagccgctgagcttccgtcttgatggagtcatcccaggctggacggagggattgaaaaacattaaaaaaggcggaaaaatcaagctggtcatccctcctgatttggcttacggaaaaacaggtgtacccgggattccggccaattcaacacttgtgtttgacgttgagttgctggatattaagccagcgccgaaagctgatgcccagccggaggcggccggagacgcaaaggcagcagatgcgaaagccgacgctaaaaag

SEQ ID NO: 42 - DNA, 699 bp, synthetic construct
  source 1..699: mol_type = other DNA
gcttttaaaaatgatgatcagcaatcggcttatgcgctcggcgcttctcttggacgctatatggaaaacagcttaaaagagcaggaaaaattaggcattgcactcgacaaaaaccagctgatcgccggcgttcaggatgcgtttgccgggaaaagcaagctaactgaccaagaaattgaacaaacattgcaaagctttgaaggacgtgtaaaaggtgccgcacaggcgaaaatggagaaagacgcgaaggaaaatacggcaaaaggggaagcgtacgctgccaaattcgcaaaggagaaggatgtgaaaaaaacagagtcaggtttactgtatttagtagaaaaagcgggcgccggagaaagtccaaaagattcagatacggttgtcgtcaattataaaggcacgctggttgacggaactgaatttgataattcttatacaagaggtgagccgctttccttccggctggacggtgtaatacccggctggacagaaggcctgaaacaagtgaagaaaggaggaaaaatcaagcttgtcattcctcctgcgcttgcttacgggcaaaacggggtgccgggaatcccagcaaattcaaccttggtgtttgaggttgaattgcttgatattaaaccggcagctaaggctgatgaaaaggcagaacagccggcggccgctgcagcagataaagcaaaagcccaa

SEQ ID NO: 43 - DNA, 693 bp, synthetic construct
  source 1..693: mol_type = other DNA
gcatttttcaaaaatgaagatcagcaatcagcttatgcgttgggtgcttctcttgcccgttatatgaataacagcctggaagaacaaaaaaagctaggtattaagcttgataaacagcagctgttagagggtgttcaggatatgtttgcagggaaatcaaaactgtctgaacagcgcatcgagcaaattttgcacggccttgagtctagagtcaaaggagcgacacaagagaaaatggaaaaggaagcgaaagaaaacgctgataagggtatagcctttgcgaataaattcgcaaaagaatcgggggtgaaaaaaaccgaaagcggattgttgtacaaaattgaaaaagaggggtccggagacccaccgcaagatgatacgactgttgtcgttcattataaaggcatgctgatcaacggaactgaatttgacaattcctatacacggggacagccgcttagtcttcatttacaaggcatcattcctggctggacagaaggcttaaagcatgtaaagaagggcggaaaaatcaagctcgtcataccacctcaacttgcttacggcaaaaacaatgtgcccggaattccgattaattcaacgttagtatttgatattgagctgctggacatcaaaacaagcccgaaaaaagatgacaaagcaagggccctcgtgacggaaatgaacaaatttaag

SEQ ID NO: 44 - DNA, 357 bp, synthetic construct
  source 1..357: mol_type = other DNA
gccggttcgctcagtgacttggaaatcggcatcataaagcggattcctgttgaagactgcctgattaaagcgatgccgggagataaagtgaaagttcattatacaggttcattgcttgaaagcggaacggtgtttgattccagctattcaaggggaagcccgattgcgtttgaattaggtgtcggccgtgtcatcaaaggctgggatcagggggtggcaggcatgtgtgtcggagaaaaaagaaagctgcaaattccatcttctcttgcttacggagagcgcggcgttcctggggtcattccgccctctgctgatttagtattcgacgtagagcttgttgatgtaaaatcagcagcc

SEQ ID NO: 45 - DNA, 429 bp, synthetic construct
  source 1..429: mol_type = other DNA
gcatctccctcggagagtgctaaaaaaaatgaaaagatatcagaagaagcgaccgtggaaagcaaagcgttcagcatttcagttgaaaaacagacgcctgatttagacggcttgatcgttgaggagctttgcatgggaaacccaaacgggaagaaagctgaaccaggtaagcgtgtctccgttcattatacaggaaagcttcaaggaaatggaaaaatctttgattctactgtaggtaaatcacggtataaatttcgccttgatgccggaaaggtgattaaaggcttagatgtcggtctcaacggcatgctagtcggcgggaaaagaaaattgacaatcccgcctgaaatggggtacggagcagaaggcgccggctccattccgccggacagctggctggtatttgacgttgagctgctgaatgtgaaa

SEQ ID NO: 46 - DNA, 471 bp, synthetic construct
  source 1..471: mol_type = other DNA
gccatcaatctcattaaaaaaggcgattatgtgaaggttgactacatacttgaagttgacggaaaagtgattgatacctctattgaagaggttgcgaaagaaaacaaaatttattatccagagcgtgaatatgaaccgatcggctttatagtcggaaacggcgagctgatcgaaggatttgaagaagcggtcatcggaatggaagtcggtgaggaaaaaacagtaacgattcctcctgaaaagggttacgggttgcgggatgaacgcttaattcaagaaatcccaaaagaaatgtttgcagacgctgacttcgagccgcaagagggcatgctgattttggccagcggcattcccgcaaaaatcattaaggtgacagatgatacagttacgcttgattttaatcatgaactagcagggaaggaattaaaattcactatcaaagtaagagatgtacagccggctgaatcagag

SEQ ID NO: 47 - DNA, 1377 bp, synthetic construct
  source 1..1377: mol_type = other DNA
gcaacagcagaggaaatgaaagcgaccgaaagtggagctcaatcggctcccttgcctatggagggggttgatatttcaccgaaacaagacgagggtgtgctcaaggtaataaaaagagagggcactggaactgaaatgccgatgatcggcgatcgtgtatttgttcactatacaggctggctgctggacgggaccaaatttgactcttctctggacaggaaagataaattttccttcgatttgggtaaaggagaagttattaaagcttgggatatagctattgcgacaatgaaggtcggcgaagtctgccatattacgtgtaaaccggaatatgcatacggttctgcaggatctcctccgaaaattccgccaaacgccacgcttgtctttgaggtagaactatttgaattcaaaggggaggatttaacagaagaggaagatggcggcatcatcagacgtatccaaaccaggggcgaaggatacgcaaaacctaatgaaggcgctattgtggaagtggcgttggaaggctactataaagacaagctgtttgatcagagagaattgcggtttgaaatcggcgagggtgaaaacttggatcttccatatggactcgagcgggcgattcagagaatggaaaaaggagagcacagcatcgtctatttgaagccatcttacgcgttcgggtccgtagggaaagagaagtttcaaattcctccgaatgctgaacttaagtatgagctgcacttaaaaagctttgaaaaagcaaaagaaagctgggagatgaattctgaagagaaactggaacaaagcacgatcgtgaaggagcgcggaacggtgtactttaaagagggaaagtacaaacaggcactgctgcagtataaaaaaattgtttcatggcttgaatatgaatcgtccttcagtaacgaagaagcgcaaaaggctcaagccttacggctcgcttcccatctaaacttagcgatgtgtcatttaaagcttcaagcgttctcagctgccattgaatcatgcaataaggcactcgaattagacagcaataatgaaaaaggtctctttagacgaggtgaagcacatcttgccgtgaatgatttcgagcttgcgcgtgctgactttcagaaagttcttcagctctatcctaacaataaagcagcaaagacgcaactggctgtctgccagcaacgtatacgccgacagctagcccgcgaaaaaaaattatatgccaatatgtttgaacgcttagcagaagaagaaaacaaagcgaaagccgaagcatcatcaggcgatcatccgacagatacagaaatgaaagaggaacaaaaatcaaacacagccggcagccagagtcaggttgaaactgaggcg

SEQ ID NO: 48 - DNA, 1110 bp, synthetic construct
  source 1..1110: mol_type = other DNA
gcaagccatccttctcctcaggccaaaccttcaaacccaagcaatccgcgtgtattttttgatgtagatataggcggagagcgcgtcggtcgtatcgttttagaattgtttgcagacatcgttccgaaaacagcggaaaatttcagagccctttgtacgggagaaaaaggcatcgggcatacgaccggaaaaccactccattttaagggatgcccgtttcacagaatcattaagaaatttatgatccagggtggagacttctctaatcaaaacggcacaggcggtgagagtatctacggcgaaaagttcgaagatgaaaactttcattataaacatgatcgagaaggattactgtccatggcgaatgccggacggaatacaaatgggtcacaattctttattactaccgtgccgacaccgcatttagatggcaaacacgttgtcttcggacaggtgattaaggggattggtgttgcaagaattctagaaaatgtagaagtaaaaggcgagaagcccgctaagttgtgcgtcattgctgaatgcggagagctcaaagaaggagatgacggaggcatttttccaaaagatggtagtggcgattcgcacccggattttcctgaagacgcggacattgatttgaaggatgttgataagattttgcttatcactgaggacttaaaaaacattggtaacacgtttttcaaaagccaaaattgggaaatggctataaaaaaatatgcagaagtgcttcgctatgtcgattcctcaaaagcggttatagaaacggctgacagggcaaagcttcagccgattgcgctgtcttgtgtgctgaatatcggcgcttgcaaacttaaaatgtcaaactggcagggggccattgacagctgtttagaagctttggagcttgatccgtctaacacaaaagcactctaccggcgcgctcaaggctggcaaggtcttaaggagtatgatcaggcactggccgatttaaaaaaagcccaagggatagctcccgaagataaggcgattcaagcagagctgctgaaagtgaaacaaaaaatcaaggcgcagaaagacaaagaaaaagcagtctatgcgaaaatgtttgcc

SEQ ID NO: 49 - DNA, 30 bp, synthetic construct
  source 1..30: mol_type = other DNA
ttgactatccatgtaggggaagcttcggct

SEQ ID NO: 50 - DNA, 30 bp, synthetic construct
  source 1..30: mol_type = other DNA
taatctattaaactagttatagggttatct

SEQ ID NO: 51 - DNA, 23 bp, synthetic construct
  source 1..23: mol_type = other DNA
cttaagtcacaatcttcaactgg

SEQ ID NO: 52 - DNA, 20 bp, synthetic construct
  source 1..20: mol_type = other DNA
tgtcctacatgaacagctta

SEQ ID NO: 53 - DNA, 52 bp, synthetic construct
  source 1..52: mol_type = other DNA
ccgttagttgaagaaggtttttatattacagcgagaatctaaggggtgaatt

SEQ ID NO: 54 - DNA, 20 bp, synthetic construct
  source 1..20: mol_type = other DNA
tcacgatcacaaaaatagcg

SEQ ID NO: 55 - DNA, 26 bp, synthetic construct
  source 1..26: mol_type = other DNA
tcttcaactaaagcacccattagttc

SEQ ID NO: 56 - DNA, 31 bp, synthetic construct
  source 1..31: mol_type = other DNA
gctgtaatataaaaaccttcttcaactaacg

SEQ ID NO: 57 - protein, 226 aa, synthetic construct
EVQLVESGGGLVQPGGSLRLSCAASGYVFTDYGMNWVRQAPGKGLEWMGWINTYIGEPIYADSVKGRFTFSLDTSKSTAYLQMNSLRAEDTAVYYCARGYRSYAMDYWGQGTLVTVSSASTKGPSVFPLAPSSKSTSGGTAALGCLVKDYFPEPVTVSWNSGALTSGVHTFPAVLQSSGLYSLSSVVTVPSSSLGTQTYICNVNHKPSNTKVDKKVEPKSCDKTHT

SEQ ID NO: 58 - protein, 214 aa, synthetic construct
DIQMTQSPSSLSASVGDRVTITCKASQNVGTNVAWYQQKPGKAPKALIYSASFLYSGVPYRFSGSGSGTDFTLTISSLQPEDFATYYCQQYNIYPLTFGQGTKVEIKRTVAAPSVFIFPPSDEQLKSGTASVVCLLNNFYPREAKVQWKVDNALQSGNSQESVTEQDSKDSTYSLSSTLTLSKADYEKHKVYACEVTHQGLSSPVTKSFNRGEC

SEQ ID NO: 59 - DNA, 1511 bp, synthetic construct
  source 1..1511: mol_type = other DNA
atgtttgcaaaacgattcaaaacctctttactgccgttattcgctggatttttattgctgtttcatttggttctggcaggaccggcggctgcgagtgctgaagttcaactggttgaatcaggcggaggcctggttcaacctggcggatcactgagactgtcatgcgcagcatcaggctatgtttttacagattatggcatgaattgggtcagacaagcacctggcaaaggcctggaatggatgggctggattaatacatatattggcgaaccgatttatgcggattcagtcaaaggcagatttacgttttcactggatacaagcaaaagcacagcatacctgcaaatgaattcactgagagcagaagatacagcggtctattattgcgcaagaggctatagatcatatgccatggattattggggacaaggcacactggttacagtttcatcagcatcaacaaaaggaccgtcagtttttccgctggcaccgtcatcaaaatcaacaagcggaggcacagcagcactgggctgcctggttaaagattattttccggaaccggttacagtcagctggaattcaggcgcactgacatcaggcgttcatacatttccggcagttctgcaatcatcaggcctgtattcactgtcatcagttgttacagttccgtcaagcagcctgggcacacaaacatatatttgcaatgtcaatcacaagccgagcaacacaaaagtcgataagaaagttgaaccgaaaagctgcgataaaacgcatacataaggaggatgacattgactaaactgaaaatgctgagtatgttaaccgtgatgattgcatctttattcattttttccagtcaggcacttgccgatatccaaatgacacaatcaccgtcatcactgtcagcatcagttggcgatagagttacaattacatgcaaagcatcacagaatgtcggcacaaatgttgcatggtatcaacaaaaaccgggaaaagcaccgaaagcactgatttattcagcaagctttctgtattcaggcgttccgtatagattttcaggctcaggcagcggcacagattttacactgacaatttcatcactgcaaccggaagattttgcgacatattattgccagcagtataacatctatccgctgacatttggccaaggcacaaaagttgaaatcaaaagaacagttgcagcaccgagcgtttttatctttccgccttcagatgaacaactgaaatcaggcacagcaagcgttgtttgcctgctgaacaacttttatccgagagaagcaaaagtccagtggaaagttgataatgcacttcaatcaggcaatagccaagaaagcgttacagaacaagatagcaaagactcaacatattcactgtcatcaacactgacactgagcaaagcggattacgaaaaacacaaagtttatgcgtgcgaagttacacatcaaggcctgtcatcaccggttacaaaatcatttaatagaggcgagtgc

SEQ ID NO: 60 - DNA, 30 bp, synthetic construct
  source 1..30: mol_type = other DNA
ttttatatagggaaaaggaggtgaactact

SEQ ID NO: 61 - DNA, 60 bp, synthetic construct
  source 1..60: mol_type = other DNA
ggtgtgaattattaggtaagctgttcatgtaggacataagaaaagtgattctgggagagc

SEQ ID NO: 62 - DNA, 63 bp, synthetic construct
  source 1..63: mol_type = other DNA
gttgaactaatgggtgctttagttgaagattagcactcgcctctattaaatgattttgtaacc

SEQ ID NO: 63 - DNA, 32 bp, synthetic construct
  source 1..32: mol_type = other DNA
taatcttcaactaaagcacccattagttcaac

SEQ ID NO: 64 - DNA, 38 bp, synthetic construct
  source 1..38: mol_type = other DNA
tttagttgaagattaggttttcacacctttctctttgg

SEQ ID NO: 65 - DNA, 21 bp, synthetic construct
  source 1..21: mol_type = other DNA
agccgaagcttcccctacatg

SEQ ID NO: 66 - DNA, 38 bp, synthetic construct
  source 1..38: mol_type = other DNA
ggggaagcttcggctgaagcaccgaaagacagcgatac

SEQ ID NO: 67 - protein, 118 aa, Escherichia coli
AEAAKPATAADSKAAFKNDDQKSAYALGASLGRYMENSLKEQEKLGIKLDKDQLIAGVQDAFADKSKLSDQEIEQTLQAFEARVKSSAQAKMEKDAADNEAKGKEYREKFAKEKGVKT

SEQ ID NO: 68 - protein, 112 aa, Escherichia coli
EAPKDSDTVVVNYKGTLIDGKEFDNSYTRGEPLSFRLDGVIPGWTEGLKNIKKGGKIKLVIPPELAYGKAGVPGIPPNSTLVFDVELLDVKPAPKADAKPEADAKAADSAKK

SEQ ID NO: 69 - protein, 224 aa, synthetic construct
QVQLQESGAEVMKPGASVKISCKATGYTFSTYWIEWVKQRPGHGLEWIGEILPGSGSTYYNEKFKGKATFTADTSSNTAYMQLSSLTSEDSAVYYCARGDGNYGYWGQGTTLTVSSASTTPPSVFPLAPGSAAQTNSMVTLGCLVKGYFPEPVTVTWNSGSLSSGVHTFPAVLQSDLYTLSSSVTVPSSPRPSETVTCNVAHPASSTKVDKKIVPRDCHHHHHH

SEQ ID NO: 70 - protein, 222 aa, synthetic construct
DIELTQSPATLSVTPGDSVSLSCRASQSISNNLHWYQQKSHESPRLLIKYVSQSSSGIPSRFSGSGSGTDFTLSINSVETEDFGMYFCQQSNSWPRTFGGGTKLEIKRADAAPTVSIFPPSSEQLTSGGASVVCFLNNFYPKDINVKWKIDGSERQNGVLNSWTDQDSKDSTYSMSSTLTLTKDEYERHNSYTCEATHKTSTSPIVKSFNRNECDYKDDDDK

SEQ ID NO: 71 - DNA, 1517 bp, synthetic construct
  source 1..1517: mol_type = other DNA
atgtttgcaaaacgattcaaaacctctttactgccgttattcgctggatttttattgctgtttcatttggttctggcaggaccggcggctgcgagtgctcaagtccaactgcaagaatcaggcgcagaagttatgaaacctggcgcatcagtcaaaatttcatgcaaagcaacaggctatacgtttagcacatattggattgagtgggttaaacaaagacctggccatggactggaatggattggcgaaattctgcctggctcaggctcaacatattacaacgaaaaattcaaaggcaaggcgacgtttacagcagatacatcatcaaatacagcgtacatgcaactgtcatcactgacatcagaagatagcgcagtttattactgcgcacgcggagatggcaattatggctattggggacaaggcacaacactgacagtttcatcagcatcaacaacaccgccttcagtttttccgctggcaccgggatcagcagcacaaacaaattcaatggttacactgggctgcctggttaaaggctattttccggaaccggttacagttacatggaattcaggctcactttcatcaggcgttcatacatttccggcagttctgcaatcagatctgtatacactgtcaagctcagttacagttccgtcatcaccgcgtccgtcagaaacagtcacatgcaatgttgcacatccggcatcatcaacaaaagtcgacaaaaaaatcgttccgagagattgccatcatcaccatcaccactaaggaggatgaaaaagatgttgatgttagcttttacatttcttttggctttgactatccatgtaggggaagcttcggctgatatcgaactgacacaatcaccggcaacactgtcagttacacctggcgattcagtttcactgtcatgcagagcatcacaaagcattagcaataacctgcattggtatcagcagaaatcacatgaaagcccgagactgctgatcaaatatgtttcacaatcatcatcaggcattccgtcaagattttcaggctcaggcagcggcacagattttacactgtcaattaatagcgtcgagacagaggattttggcatgtatttttgccaacaatcaaatagctggccgagaacatttggcggaggcacaaaactggaaattaaacgcgcagatgcagcaccgacagtttcaatttttccgccttcatcagaacaactgacatcaggcggagcatcagttgtttgctttctgaataacttttacccgaaggacatcaacgtcaaatggaaaattgatggcagcgaaagacaaaatggcgttctgaattcatggacagatcaggattcaaaagatagcacgtattcaatgtcaagcacactgacactgacgaaagatgaatatgaacgccataacagctatacatgcgaagcgacacataaaacatcaacaagcccgattgtcaaaagctttaatcgcaatgaatgcgactataaagacgacgacgacaaa

SEQ ID NO: 72 - DNA, 21 bp, synthetic construct
  source 1..21: mol_type = other DNA
cacaagccctgcatgatcaaa

SEQ ID NO: 73 - DNA, 19 bp, synthetic construct
  source 1..19: mol_type = other DNA
tcaggattgttactgcgaa

SEQ ID NO: 74 - DNA, 52 bp, synthetic construct
  source 1..52: mol_type = other DNA
ccgttagttgaagaaggtttttatattacagccgggtcgttttatttgtttg

SEQ ID NO: 75 - DNA, 20 bp, synthetic construct
  source 1..20: mol_type = other DNA
gataagtatgatgctcacca

SEQ ID NO: 76 - DNA, 56 bp, synthetic construct
  source 1..56: mol_type = other DNA
ggttttgcctgctttcgcagtaacaatcctgataagaaaagtgattctgggagagc

SEQ ID NO: 77 - DNA, 32 bp, synthetic construct
  source 1..32: mol_type = other DNA
agtagttcacctccttttccctatataaaagc

SEQ ID NO: 78 - DNA, 124 bp, synthetic construct
  source 1..124: mol_type = other DNA
gcttttatatagggaaaaggaggtgaactactatgaaaaagatgttgatgttagcttttacatttcttttggctttgactatccatgtaggggaagcttcggctgctgaagctgcaaaacctgc

SEQ ID NO: 79 - DNA, 53 bp, synthetic construct
  source 1..53: mol_type = other DNA
gttgaactaatgggtgctttagttgaagattattttttagcagaatctgcggc

SEQ ID NO: 80 - DNA, 124 bp, synthetic construct
  source 1..124: mol_type = other DNA
gcttttatatagggaaaaggaggtgaactactatgagacaagggctgatggcagcagtactttttgcgacctttgctttaacgggatgcggaacggattcagccgctgaagctgcaaaacctgc

SEQ ID NO: 81 - protein, 270 aa, Escherichia coli
MKSLFKVTLLATTMAVALHAPITFAAEAAKPATAADSKAAFKNDDQKSAYALGASLGRYMENSLKEQEKLGIKLDKDQLIAGVQDAFADKSKLSDQEIEQTLQAFEARVKSSAQAKMEKDAADNEAKGKEYREKFAKEKGVKTSSTGLVYQVVEAGKGEAPKDSDTVVVNYKGTLIDGKEFDNSYTRGEPLSFRLDGVIPGWTEGLKNIKKGGKIKLVIPPELAYGKAGVPGIPPNSTLVFDVELLDVKPAPKADAKPEADAKAADSAKK

SEQ ID NO: 82 - protein, 273 aa, Lelliottia amnigena
MKSLFKVTLLATTMAVALNAPLSFAADTVAKPAASADSKAAFKNDDQKSAYALGASLGRYMENSLKEQEKLGIKLDKDQLIAGVQDAFADKSKLSDQEIEQTLQAFEARVKGAAQGKMEKDAKDNEAKGKAYRDTFAKEKGVKTSSTGLLYKVEKAGTGDAPKDSDTVVVNYKGTLIDGKEFDNSYTRGEPLSFRLDGVIPGWTEGLKNIKKGGKIQLVIPPDLAYGKTGVPGIPANSTLVFDVELLDIKPAPKADAKSAAAEDDKAADAAKK

SEQ ID NO: 83 - protein, 276 aa, Klebsiella quasipneumoniae
MKSLFKVTLLATTMAVALNAPLTFAADTAAKAAPAAESKSAFKNDDQKSAYALGASLGRYMENSLKEQEKLGIKLDKAQLIAGVQDAFADKSKLSDQEIEQTLQAFETRVKTAAQQKMQNHATENETKGKAFRDSFAKEKGVKTSKTGLLYKVEKEGTGDAPKDSDTVVVNYKGTLIDGKEFDNSYTRGEPLSFRLDGVIPGWTEGLKNIKKGGKIKLVIPPDLAYGKTGVPGIPANSTLVFDVELLDIKPAPKADAQPEAAGDAKAADAKADAKK

SEQ ID NO: 84 - protein, 274 aa, Erwinia sp. B116
MKSLFKVTLLATTLAAAFTAPLAIAADAAAAPAAQQAPKNAAFKNDDQQSAYALGASLGRYMENSLKEQEKLGIALDKNQLIAGVQDAFAGKSKLTDQEIEQTLQSFEGRVKGAAQAKMEKDAKENTAKGEAYAAKFAKEKDVKKTESGLLYLVEKAGAGESPKDSDTVVVNYKGTLVDGTEFDNSYTRGEPLSFRLDGVIPGWTEGLKQVKKGGKIKLVIPPALAYGQNGVPGIPANSTLVFEVELLDIKPAAKADEKAEQPAAAAADKAKAQ

SEQ ID NO: 85 - protein, 276 aa, Pantoea sp. Nvir
MKSLFKVTTLATIISIMLHAKLTAASTELTRASDTKDTVSQISKNTFFKNEDQQSAYALGASLARYMNNSLEEQKKLGIKLDKQQLLEGVQDMFAGKSKLSEQRIEQILHGLESRVKGATQEKMEKEAKENADKGIAFANKFAKESGVKKTESGLLYKIEKEGSGDPPQDDTTVVVHYKGMLINGTEFDNSYTRGQPLSLHLQGIIPGWTEGLKHVKKGGKIKLVIPPQLAYGKNNVPGIPINSTLVFDIELLDIKTSPKKDDKARALVTEMNKFK

SEQ ID NO: 86 - protein, 157 aa, Methanococcus jannaschii
LINLIKKGDYVKVDYILEVDGKVIDTSIEEVAKENKIYYPEREYEPIGFIVGNGELIEGFEEAVIGMEVGEEKTVTIPPEKGYGLRDERLIQEIPKEMFADADFEPQEGMLILASGIPAKIIKVTDDTVTLDFNHELAGKELKFTIKVRDVQPAESE

SEQ ID NO: 87 - protein, 428 aa, Escherichia coli
MKNWKTLLLGIAMIANTSFAAPQVVDKVAAVVNNGVVLESDVDGLMQSVKLNAAQARQQLPDDATLRHQIMERLIMDQIILQMGQKMGVKISDEQLDQAIANIAKQNNMTLDQMRSRLAYDGLNYNTYRNQIRKEMIISEVRNNEVRRRITILPQEVESLAQQVGNQNDASTELNLSHILIPLPENPTSDQVNEAESQARAIVDQARNGADFGKLAIAHSADQQALNGGQMGWGRIQELPGIFAQALSTAKKGDIVGPIRSGVGFHILKVNDLRGESKNISVTEVHARHILLKPSPIMTDEQARVKLEQIAADIKSGKTTFAAAAKEFSQDPGSANQGGDLGWATPDIFDPAFRDALTRLNKGQMSAPVHSSFGWHLIELLDTRNVDKTDAAQKDRAYRMLMNRKFSEEAASWMQEQRASAYVKILSN

SEQ ID NO: 88 - protein, 190 aa, Escherichia coli
MFKSTLAAMAAVFALSALSPAAMAAKGDPHVLLTTSAGNIELELDKQKAPVSVQNFVDYVNSGFYNNTTFHRVIPGFMIQGGGFTEQMQQKKPNPPIKNEADNGLRNTRGTIAMARTADKDSATSQFFINVADNAFLDHGQRDFGYAVFGKVVKGMDVADKISQVPTHDVGPYQNVPSKPVVILSAKVLP

SEQ ID NO: 89 - protein, 432 aa, Escherichia coli
MQVSVETTQGLGRRVTITIAADSIETAVKSELVNVAKKVRIDGFRKGKVPMNIVAQRYGASVRQDVLGDLMSRNFIDAIIKEKINPAGAPTYVPGEYKLGEDFTYSVEFEVYPEVELQGLEAIEVEKPIVEVTDADVDGMLDTLRKQQATWKEKDGAVEAEDRVTIDFTGSVDGEEFEGGKASDFVLAMGQGRMIPGFEDGIKGHKAGEEFTIDVTFPEEYHAENLKGKAAKFAINLKKVEERELPELTAEFIKRFGVEDGSVEGLRAEVRKNMERELKSAIRNRVKSQAIEGLVKANDIDVPAALIDSEIDVLRRQAAQRFGGNEKQALELPRELFEEQAKRRVVVGLLLGEVIRTNELKADEERVKGLIEEMASAYEDPKEVIEFYSKNKELMDNMRNVALEEQAVEAVLAKAKVTEKETTFNELMNQQA

SEQ ID NO: 90 - protein, 135 aa, Saccharomyces cerevisiae
MMFNIYLFVTFFSTILAGSLSDLEIGIIKRIPVEDCLIKAMPGDKVKVHYTGSLLESGTVFDSSYSRGSPIAFELGVGRVIKGWDQGVAGMCVGEKRKLQIPSSLAYGERGVPGVIPPSADLVFDVELVDVKSAA

SEQ ID NO: 91 - protein, 143 aa, Arabidopsis thaliana
MSPSESAKKNEKISEEATVESKAFSISVEKQTPDLDGLIVEELCMGNPNGKKAEPGKRVSVHYTGKLQGNGKIFDSTVGKSRYKFRLDAGKVIKGLDVGLNGMLVGGKRKLTIPPEMGYGAEGAGSIPPDSWLVFDVELLNVK

SEQ ID NO: 92 - protein, 459 aa, Homo sapiens
MTAEEMKATESGAQSAPLPMEGVDISPKQDEGVLKVIKREGTGTEMPMIGDRVFVHYTGWLLDGTKFDSSLDRKDKFSFDLGKGEVIKAWDIAIATMKVGEVCHITCKPEYAYGSAGSPPKIPPNATLVFEVELFEFKGEDLTEEEDGGIIRRIQTRGEGYAKPNEGAIVEVALEGYYKDKLFDQRELRFEIGEGENLDLPYGLERAIQRMEKGEHSIVYLKPSYAFGSVGKEKFQIPPNAELKYELHLKSFEKAKESWEMNSEEKLEQSTIVKERGTVYFKEGKYKQALLQYKKIVSWLEYESSFSNEEAQKAQALRLASHLNLAMCHLKLQAFSAAIESCNKALELDSNNEKGLFRRGEAHLAVNDFELARADFQKVLQLYPNNKAAKTQLAVCQQRIRRQLAREKKLYANMFERLAEEENKAKAEASSGDHPTDTEMKEEQKSNTAGSQSQVETEA

SEQ ID NO: 93 - protein, 370 aa, Homo sapiens
MSHPSPQAKPSNPSNPRVFFDVDIGGERVGRIVLELFADIVPKTAENFRALCTGEKGIGHTTGKPLHFKGCPFHRIIKKFMIQGGDFSNQNGTGGESIYGEKFEDENFHYKHDREGLLSMANAGRNTNGSQFFITTVPTPHLDGKHVVFGQVIKGIGVARILENVEVKGEKPAKLCVIAECGELKEGDDGGIFPKDGSGDSHPDFPEDADIDLKDVDKILLITEDLKNIGNTFFKSQNWEMAIKKYAEVLRYVDSSKAVIETADRAKLQPIALSCVLNIGACKLKMSNWQGAIDSCLEALELDPSNTKALYRRAQGWQGLKEYDQALADLKKAQGIAPEDKAIQAELLKVKQKIKAQKDKEKAVYAKMFA

SEQ ID NO: 94 - DNA, 575 bp, Bacillus sp. KSM-S237
  source 1..575: mol_type = genomic DNA
gatttgccgatgcaacaggcttatatttagaggaaatttctttttaaattgaatacggaataaaatcaggtaaacaggtcctgattttatttttttgagttttttagagaactgaagattgaaataaaagtagaagacaaaggacataagaaaattgcattagttttaattatagaaaacgcctttttataattatttatacctagaacgaaaatactgtttcgaaagcggtttactataaaaccttatattccggctcttttttaaaacagggggtaaaaattcactctagtattctaatttcaacatgctataataaatttgtaagacgcaatatgcatctctttttttacgatatatgtaagcggttaaccttgtgctatatgccgatttaggaaggggggtagattgagtcaagtagtaataatatagataacttataagttgttgagaagcaggagagcatctgggttactcacaagtttttttaaaactttaacgaaagcactttcggtaatgcttatgaatttagctatttgattcaattactttaaaaatatttaggaggtaatatg

SEQ ID NO: 95 - DNA, 617 bp, Bacillus sp. KSM-64
  source 1..617: mol_type = genomic DNA
gaacaagtacttaccattttagagtcaaaagatagaagccaagcaggatttgccgatgcaaccggcttatatttagagggaatttctttttaaattgaatacggaataaaatcaggtaaacaggtcctgattttatttttttgaatttttttgagaactaaagattgaaatagaagtagaagacaacggacataagaaaattgtattagttttaattatagaaaacgcttttctataattatttatacctagaacgaaaatactgtttcgaaagcggtttactataaaaccttatattccggctctttttttaaacagggggtgaaaattcactctagtattctaatttcaacatgctataataaatttgtaagacgcaatatacatcttttttttatgatatttgtaagcggttaaccttgtgctatatgccgatttaggaagggggtagattgagtcaagtagtcataatttagataacttataagttgttgagaagcaggagagaatctgggttactcacaagttttttaaaacattatcgaaagcactttcggttatgcttatgaatttagctatttgattcaattactttaataattttaggaggtaatatg

SEQ ID NO: 96 - DNA, 193 bp, Bacillus subtilis
  source 1..193: mol_type = genomic DNA
taagaaaagtgattctgggagagccgggatcacttttttatttaccttatgcccgaaatgaaagctttatgacctaattgtgtaactatatcctattttttcaaaaaatattttaaaaacgagcaggatttcagaaaaaatcgtggaattgatacactaatgcttttatatagggaaaaggtggtgaactact

SEQ ID NO: 97 - DNA, 87 bp, Bacillus sp. KSM-S237
  source 1..87: mol_type = genomic DNA
atgttaagaaagaaaacaaagcagttgatttcttccattcttattttagttttacttctatctttatttccggcagctcttgcagca

SEQ ID NO: 98 - DNA, 87 bp, Bacillus sp. KSM-64
  source 1..87: mol_type = genomic DNA
atgttaagaaagaaaacaaagcagttgatttcttccattcttattttagttttacttctatctttatttccgacagctcttgcagca

SEQ ID NO: 99 - DNA, 74 bp, Bacillus subtilis
  source 1..74: mol_type = genomic DNA
atgtttgcaaaacgattcaaaacctctttactgccgttattcgctggatttttattgctgtttcatttggttct

SEQ ID NO: 100 - protein, 104 aa, Aspergillus oryzae
ACDYTCGSNCYSSSDVSTAQAAGYQLHEDGETVGSNSYPHKYNNYEGFDFSVSSPYYEWPILSSGDVYSGGSPGADRVVFNENNQLAGVITHTGASGNNFVECT

SEQ ID NO: 101 - DNA, 312 bp, synthetic construct
  source 1..312: mol_type = other DNA
gcttgtgattatacatgcggatcaaactgctactcaagttctgatgtatcaaccgcgcaagcggcaggctatcagctgcatgaggacggagaaacagtcggctcaaattcttatccgcataaatacaacaactatgagggctttgatttttctgtttccagtccttattatgaatggccgattttatcgtccggtgatgtgtacagcggcggaagcccaggggctgacagagtggtatttaatgaaaataatcaacttgccggtgtcatcactcacacgggggcaagcggaaacaatttcgttgaatgtacg